European Patent Specification EP 3 659 609 B1, published May 8, 2024. Title: THERAPEUTIC AGENT FOR FIBROSIS. Applicant: Kyorin pharmaceutical co.,ltd. The sequence listing filed with the application follows.

SEQUENCE LISTING (61 sequences)

SEQ ID NO: 1 - RNA, 15 nt, Artificial
  Synthetic RNA
agagguuguuggaac

SEQ ID NO: 2 - RNA, 15 nt, Artificial
  Synthetic RNA
ccuugacacaguccu

SEQ ID NO: 3 - RNA, 15 nt, Artificial
  Synthetic RNA
cgugaaugcaugugc

SEQ ID NO: 4 - RNA, 15 nt, Artificial
  Synthetic RNA
ggagaagagauucau

SEQ ID NO: 5 - RNA, 15 nt, Artificial
  Synthetic RNA
guauccgaugucagg

SEQ ID NO: 6 - RNA, 15 nt, Artificial
  Synthetic RNA
guuccaacaaccucu

SEQ ID NO: 7 - RNA, 15 nt, Artificial
  Synthetic RNA
aggacugugucaagg

SEQ ID NO: 8 - RNA, 15 nt, Artificial
  Synthetic RNA
gcacaugcauucacg

SEQ ID NO: 9 - RNA, 15 nt, Artificial
  Synthetic RNA
augaaucucuucucc

SEQ ID NO: 10 - RNA, 15 nt, Artificial
  Synthetic RNA
ccugacaucggauac

SEQ ID NO: 11 - RNA, 19 nt, Artificial
  Synthetic RNA
agagguuguuggaacuccc

SEQ ID NO: 12 - RNA, 19 nt, Artificial
  Synthetic RNA
ccuugacacaguccugccu

SEQ ID NO: 13 - RNA, 19 nt, Artificial
  Synthetic RNA
cgugaaugcaugugcucca

SEQ ID NO: 14 - RNA, 19 nt, Artificial
  Synthetic RNA
ggagaagagauucaucuua

SEQ ID NO: 15 - RNA, 19 nt, Artificial
  Synthetic RNA
guauccgaugucaggucuc

SEQ ID NO: 16 - RNA, 21 nt, Artificial
  Synthetic RNA
agagguuguuggaacucccuc

SEQ ID NO: 17 - RNA, 21 nt, Artificial
  Synthetic RNA
ccuugacacaguccugccucg

SEQ ID NO: 18 - RNA, 21 nt, Artificial
  Synthetic RNA
cgugaaugcaugugcuccacg

SEQ ID NO: 19 - RNA, 21 nt, Artificial
  Synthetic RNA
ggagaagagauucaucuuauc

SEQ ID NO: 20 - RNA, 21 nt, Artificial
  Synthetic RNA
guauccgaugucaggucucug

SEQ ID NO: 21 - RNA, 23 nt, Artificial
  Synthetic RNA
agagguuguuggaacucccucca

SEQ ID NO: 22 - RNA, 23 nt, Artificial
  Synthetic RNA
ccuugacacaguccugccucgcc

SEQ ID NO: 23 - RNA, 23 nt, Artificial
  Synthetic RNA
cgugaaugcaugugcuccacggc

SEQ ID NO: 24 - RNA, 23 nt, Artificial
  Synthetic RNA
ggagaagagauucaucuuaucuc

SEQ ID NO: 25 - RNA, 23 nt, Artificial
  Synthetic RNA
guauccgaugucaggucucuggu

SEQ ID NO: 26 - RNA, 25 nt, Artificial
  Synthetic RNA
ggagagguuguuggaacucccucca

SEQ ID NO: 27 - RNA, 25 nt, Artificial
  Synthetic RNA
ggccuugacacaguccugccucgcc

SEQ ID NO: 28 - RNA, 25 nt, Artificial
  Synthetic RNA
ggcgugaaugcaugugcuccacggc

SEQ ID NO: 29 - RNA, 25 nt, Artificial
  Synthetic RNA
ggggagaagagauucaucuuaucuc

SEQ ID NO: 30 - RNA, 25 nt, Artificial
  Synthetic RNA
ggguauccgaugucaggucucuggu

SEQ ID NO: 31 - RNA, 48 nt, Artificial
  Synthetic RNA
gagggaguuccaacaaccucuccggagagguuguuggaacucccucca

SEQ ID NO: 32 - RNA, 48 nt, Artificial
  Synthetic RNA
cgaggcaggacugugucaaggccggccuugacacaguccugccucgcc

SEQ ID NO: 33 - RNA, 48 nt, Artificial
  Synthetic RNA
cguggagcacaugcauucacgccggcgugaaugcaugugcuccacggc

SEQ ID NO: 34 - RNA, 48 nt, Artificial
  Synthetic RNA
gauaagaugaaucucuucuccccggggagaagagauucaucuuaucuc

SEQ ID NO: 35 - RNA, 48 nt, Artificial
  Synthetic RNA
cagagaccugacaucggauacccggguauccgaugucaggucucuggu

SEQ ID NO: 36 - RNA, 25 nt, Artificial
  Synthetic RNA
ggcuuuucgaucuggaaguccgcca

SEQ ID NO: 37 - RNA, 25 nt, Artificial
  Synthetic RNA
ggucuuuucgaucuggaaguccgcc

SEQ ID NO: 38 - RNA, 25 nt, Artificial
  Synthetic RNA
ggcuucuuuucgaucuggaaguccg

SEQ ID NO: 39 - RNA, 25 nt, Artificial
  Synthetic RNA
gggaagagauucaucuuaucuccau

SEQ ID NO: 40 - RNA, 25 nt, Artificial
  Synthetic RNA
ggagauucaucuuaucuccauagaa

SEQ ID NO: 41 - RNA, 23 nt, Artificial
  Synthetic RNA
gcggacuuccagaucgaaaagcc

SEQ ID NO: 42 - RNA, 23 nt, Artificial
  Synthetic RNA
cggacuuccagaucgaaaagacc

SEQ ID NO: 43 - RNA, 23 nt, Artificial
  Synthetic RNA
gacuuccagaucgaaaagaagcc

SEQ ID NO: 44 - RNA, 23 nt, Artificial
  Synthetic RNA
ggagauaagaugaaucucuuccc

SEQ ID NO: 45 - RNA, 23 nt, Artificial
  Synthetic RNA
cuauggagauaagaugaaucucc

SEQ ID NO: 46 - RNA, 48 nt, Artificial
  Synthetic RNA
ggagauaagaugaaucucuucccgggaagagauucaucuuaucuccau

SEQ ID NO: 47 - RNA, 48 nt, Artificial
  Synthetic RNA
cuauggagauaagaugaaucuccggagauucaucuuaucuccauagaa

SEQ ID NO: 48 - RNA, 48 nt, Artificial
  Synthetic RNA
gcggacuuccagaucgaaaagccggcuuuucgaucuggaaguccgcca

SEQ ID NO: 49 - RNA, 48 nt, Artificial
  Synthetic RNA
cggacuuccagaucgaaaagaccggucuuuucgaucuggaaguccgcc

SEQ ID NO: 50 - RNA, 48 nt, Artificial
  Synthetic RNA
gacuuccagaucgaaaagaagccggcuucuuuucgaucuggaaguccg

SEQ ID NO: 51 - RNA, 19 nt, Artificial
  Synthetic RNA
cuguccucggccuaucuuc

SEQ ID NO: 52 - RNA, 19 nt, Artificial
  Synthetic RNA
uauuugggugguucaguug

SEQ ID NO: 53 - RNA, 19 nt, Artificial
  Synthetic RNA
caacuccagcacaauguuc

SEQ ID NO: 54 - RNA, 19 nt, Artificial
  Synthetic RNA
uacuugaucaucugcgaga

SEQ ID NO: 55 - RNA, 24 nt, Artificial
  Synthetic RNA
aaguacuuccauacuguccucucc

SEQ ID NO: 56 - DNA, 942 bp, Homo sapiens
atggcaggacagcccggccacatgccccatggagggagttccaacaacctctgccacaccctggggcctgtgcatcctcctgacccacagaggcatcccaacacgctgtcttttcgctgctcgctggcggacttccagatcgaaaagaagataggccgaggacagttcagcgaggtgtacaaggccacctgcctgctggacaggaagacagtggctctgaagaaggtgcagatctttgagatgatggacgccaaggcgaggcaggactgtgtcaaggagatcggcctcttgaagcaactgaaccacccaaatatcatcaagtatttggactcgtttatcgaagacaacgagctgaacattgtgctggagttggctgacgcaggggacctctcgcagatgatcaagtactttaagaagcagaagcggctcatcccggagaggacagtatggaagtactttgtgcagctgtgcagcgccgtggagcacatgcattcacgccgggtgatgcaccgagacatcaagcctgccaacgtgttcatcacagccacgggcgtcgtgaagctcggtgaccttggtctgggccgcttcttcagctctgagaccaccgcagcccactccctagtggggacgccctactacatgtcaccggagaggatccatgagaacggctacaacttcaagtccgacatctggtccctgggctgtctgctgtacgagatggcagccctccagagccccttctatggagataagatgaatctcttctccctgtgccagaagatcgagcagtgtgactaccccccactccccggggagcactactccgagaagttacgagaactggtcagcatgtgcatctgccctgacccccaccagagacctgacatcggatacgtgcaccaggtggccaagcagatgcacatctggatgtccagcacctga

SEQ ID NO: 57 - DNA, 25 bp, Artificial
  Synthetic DNA
attggagggcaagtctggtgccagc

SEQ ID NO: 58 - DNA, 21 bp, Artificial
  Synthetic DNA
cggctaccacatccaaggaag

SEQ ID NO: 59 - DNA, 18 bp, Artificial
  Synthetic DNA
gctggaattaccgcggct

SEQ ID NO: 60 - DNA, 48 bp, Artificial
  Synthetic DNA
agtatgtctagactgaagtatgtctagactgaagtatgtctagactga

SEQ ID NO: 61 - RNA, 48 nt, Artificial
  Synthetic RNA
gacucguuuaucgaagacaacccggguugucuucgauaaacgagucca